European Patent Application EP 4 353 745 A1, published April 17, 2024. Title: A GROUP OF B7H3 MONOCLONAL ANTIBODIES AND MEDICAL USE THEREOF. Applicant: Innolake Pharmaceuticals (Hangzhou) Co., Ltd. The sequence listing filed with the application follows.

SEQUENCE LISTING (124 sequences)

SEQ ID NO: 1 - protein, 119 aa, artificial
EVQLQQSGAELVRPGALVKLSCKTSGFNIKAYYIHWVKQRPEQGLEWIGWIDPENGNTFYDPKFQGKASITADTSSNTAYLQLSSLTSEDAAVYYCTRSSTRLRPFDYWGQGTTLTVSS

SEQ ID NO: 2 - protein, 111 aa, artificial
DIVMTQAAFSNPVTLGTSASISCRSSKSLLHSNGITYLYWYLQKSGQSPQLLIYQMSNLASGVPDRFSSSGSGTDFTLRISRVEAEDVGVYYCAQNLELYTFGGGTKLEIK

SEQ ID NO: 3 - protein, 118 aa, artificial
EVQLQQSGPELVKPGASVKISCKTSGYTFTEYTIHWVKQSHGKSLEWIGGINPNSGGTTYNLKFKGKATLTVDKSSSTVYMELRSLTSEDSAVYYCARKEGFFTTDYWGQGTTLTVSS

SEQ ID NO: 4 - protein, 106 aa, artificial
QTVLTQSPAIMSASPGEKVTMTCSASSSLSYIHWYRQKSGTSPKRWIYDTSNLATGVPVRFSGSGSGTSYSLTISSMEAEDAATYYCQQWHYNPPTFGGGTKLEIK

SEQ ID NO: 5 - protein, 121 aa, artificial
QVQLQQSGAELARPGASVKMSCKTSGYTFITYTIHWVKQRPGQGLEWIGYINPTSDYANFNQKFKDKATLTADKSSRTAYMQLSSLTSEDSAVYYCARWGTTVFQFYFDYWGQGTTLTVSS

SEQ ID NO: 6 - protein, 106 aa, artificial
QIVLSQSPAILSASPGEKVTMTCRASQSLSYINWYQLKPGSSPKPWIYATSSLQSGVPARFSGSASGTSYSLTISRVEAEDAATYFCQHWSSDPPTIGGGTKLEIK

SEQ ID NO: 7 - protein, 119 aa, artificial
EVQLQQSGTELVRPGALVKLSCKASALNIKDFYMHWVKQRPERGLEWIGWIDPDNGNTIYDPKFQGKASITADISSSTAYLQLSSLTSEDTAVYYCARSSTRQRPFDYWGQGTTLTVSS

SEQ ID NO: 8 - protein, 107 aa, artificial
DIVMTQSHKVMSTSVGDRVSITCKASQDVRTGVAWYQQKPGQSPKLLIYSAFYRYTGVPDRFTVSGSGADFTFTITSVQAEDLAVYYCQQYYSIPWTFGGGTKLEIK

SEQ ID NO: 9 - protein, 118 aa, artificial
EVQLQQSGPELVKPGASVKISCKTSGYTFTEYIMHWVKQSRGKSLEWIGGINPNSGGTTYNEKFKGKATLTVDKSASTAYMELRSLTSEDSAIYYCARRMPYWYFDVWGAGTTVTVSS

SEQ ID NO: 10 - protein, 106 aa, artificial
QIVLTQSPAIMSASPGEKVTMTCSASSSVSYIHWYRQKSGTSPKRWVYDTSKLASGVPARFSGSGSGTSYSLTISSMEAEDAATYYCQQWVSNPLTFGAGTKLELK

SEQ ID NO: 11 - protein, 120 aa, artificial
EVQLQQSGPELVKPGASVKLSCKTSGYTFTEYIMHWVKQSHGKSLEWIGGINPNTGGITYNQKFKDKATLTVDKSSSTAYMELRSLTSDDSAVYFSARAGGNFLWYFDVWGAGTTVTVSS

SEQ ID NO: 12 - protein, 106 aa, artificial
QIVLTQSPATMSASPGEKVTMTCSASSSVSYMHWYQQKSDMSPKRWLYDTSKLASGVPARFSGSGSGTSYSLAISSMEAEDAATYYCQQWNSNPLTFGTGTKLELK

SEQ ID NO: 13 - protein, 114 aa, artificial
QVQLQQSGPEVVKPGALVRISCKASGYTFTSYDINWVKQRPGQGLEWIGWIDPGDGSTKYNEKFKGKATLTADKSSSTAYMQFSSLTSENSAVYFCVRRGFDYWGQGTTLTVSS

SEQ ID NO: 14 - protein, 106 aa, artificial
QILLTQSPAIMSASPGEKVTMTCRTSSSVSYLHWFQQKPGSSPKLWIHDTSNLASGFPARFSGSGSGTSYSLIISSMEAEDAATYYCHQRSSYPWTFGGGTKLEIK

SEQ ID NO: 15 - protein, 118 aa, artificial
EVKLVESGGGLVRPGGSLKLSCAASGFTFSSYAVSWVRQTPEKRLEWVASISGGGIYIYYPDSVKGRFTISRDNAKNNLYLQMNSLTPDDTALYYCARHGGAGYFDYWGQGTTLTVSS

SEQ ID NO: 16 - protein, 108 aa, artificial
DSLMTQSPASLSASVGETVTITCRGSESVHSYLAWYQQKQGKSPQLLVYNAKTLQSGVPSRFSGSGSGTQFSLRINSLQPEDFGTYYCQQHYGSPPWTFGGGTILEIK

SEQ ID NO: 17 - protein, 126 aa, artificial
QVQLQQSGPELVRPGVSVKISCKGSGYTFTDYAMHWVKQSHAKSLEWIGVINSYYGNTHYNQKFKGKATMTVDKSSSTAYMELARLTSEDSAIYYCARAGGYSYGSSYRPDRFAYWGQGTLVIVSA

SEQ ID NO: 18 - protein, 107 aa, artificial
DIQMTQSPASQSASLGESVTITCLASQTIGTWLAWYQQKPGKSPQLLIYAATNLADGVPSRFSGSGSGTKFSFKISSLQAEDFVSYYCQQLYSTPYTFGGGTKLEIK

SEQ ID NO: 19 - protein, 121 aa, artificial
EVQLQQSGPELVKPGASVKISCKTSGYTFTEYTMHWVKQSHGKNLEWIGGINTDNGGTTYSQKFKDKATLTVDRSSSTAYMVLRSLTSEDSAVYYCARSFNNYGPAWFAYWGQGALVTVSA

SEQ ID NO: 20 - protein, 106 aa, artificial
DIVMTQSHKFMSTSIGDRVSITCKASQDVRSAVAWYQQRPGQSPKLLIYWASTRHTGVPARFTGSGSGTDYTLTINNVQSEDLAGYFCQQYSSYFTFGGGTKLEKK

SEQ ID NO: 21 - protein, 121 aa, artificial
EVQLQQSGPELVKSGASVNISCKTSGYTFTENTMHWVKLSHGKSLEWIGGINPNNGGTTYNQKFKGKATLTVDKSSSTAYMELRSLTSEDSAVYYCARRGRWPPDWYFDVWGAGTTVTVSS

SEQ ID NO: 22 - protein, 106 aa, artificial
QIVLTQSPAIMSASPGEKVTMTCSASSSLSYMHWYQQKSGTSPKRWIYDTSKLASGVPARFSGSGSGTSYSLTISSMEAEDAATYYCQQWSSNPLTFGAGTKLELK

SEQ ID NO: 23 - protein, 120 aa, artificial
QVQLQQPGAELVKPGASVKLSCKASGYTFTSYYIYWLKQRPGQGLEWIGGIKPSNGDTNFNAKFMNKATLTVDKSSSTAYMQLSSLTSEDSAIYYCTRFFYGSPYDFDVWGAGTTVTVSS

SEQ ID NO: 24 - protein, 107 aa, artificial
NIVMTQSPKSMSMAVGERVTLTCKASENVDTHVSWYQQKPEQSPTLLMYGTSNRFTGVPDRFTGSGSATDFTLTISSVQAEDLADYHCGQSYRYPYTFGGGTKLEIK

SEQ ID NO: 25 - protein, 120 aa, artificial
EVQLQQSGPELVKPGASVKISCKTSGYTFTEYVMHWVKQRHGQSLEWIGGINPNTGGTTYNQKFEGKATLTVDKSSSSAYMEFRSLTSEDSAVYYCARRMPFGISAMDYWGQGTSVTVSS

SEQ ID NO: 26 - protein, 106 aa, artificial
QIVLTQSPAIMSASPGEKVTMTCSASSSVSYIHWFQQKSGTSPKRWISETSKLASGVPARFSGSGSGTSYSLTISSMGAEDAATYYCHQWISYPPTFGAGTKLELK

SEQ ID NO: 27 - protein, 123 aa, artificial
QVQLQQSGPELVRPGVSVKISCKGSGYTFTDHAIHWVKQSHAKSLEWIGVINTYSGNTNFNQKLKGKATMTVDKSSSTAYMELARLTSEDSAIYYCARGAHSSGYPYWYFDVWGAGTTVTVSS

SEQ ID NO: 28 - protein, 106 aa, artificial
QIVLSQSPAILSASAGEKVTMTCRASSSVSYMHWYQQKPGSSPKPWIYATSNLASGVPARFSGSGSGTSYSLTISRVEAEDAATYYCQQWSTNPFTFGSGTKLEMK

SEQ ID NO: 29 - protein, 5 aa, artificial
AYYIH

SEQ ID NO: 30 - protein, 17 aa, artificial
WIDPENGNTFYDPKFQG

SEQ ID NO: 31 - protein, 10 aa, artificial
SSTRLRPFDY

SEQ ID NO: 32 - protein, 16 aa, artificial
RSSKSLLHSNGITYLY

SEQ ID NO: 33 - protein, 7 aa, artificial
QMSNLAS

SEQ ID NO: 34 - protein, 8 aa, artificial
AQNLELYT

SEQ ID NO: 35 - protein, 5 aa, artificial
EYTIH

SEQ ID NO: 36 - protein, 17 aa, artificial
GINPNSGGTTYNLKFKG

SEQ ID NO: 37 - protein, 9 aa, artificial
KEGFFTTDY

SEQ ID NO: 38 - protein, 10 aa, artificial
SASSSLSYIH

SEQ ID NO: 39 - protein, 7 aa, artificial
DTSNLAT

SEQ ID NO: 40 - protein, 9 aa, artificial
QQWHYNPPT

SEQ ID NO: 41 - protein, 5 aa, artificial
TYTIH

SEQ ID NO: 42 - protein, 17 aa, artificial
YINPTSDYANFNQKFKD

SEQ ID NO: 43 - protein, 12 aa, artificial
WGTTVFQFYFDY

SEQ ID NO: 44 - protein, 10 aa, artificial
RASQSLSYIN

SEQ ID NO: 45 - protein, 7 aa, artificial
ATSSLQS

SEQ ID NO: 46 - protein, 9 aa, artificial
QHWSSDPPT

SEQ ID NO: 47 - protein, 5 aa, artificial
DFYMH

SEQ ID NO: 48 - protein, 17 aa, artificial
WIDPDNGNTIYDPKFQG

SEQ ID NO: 49 - protein, 10 aa, artificial
SSTRQRPFDY

SEQ ID NO: 50 - protein, 11 aa, artificial
KASQDVRTGVA

SEQ ID NO: 51 - protein, 7 aa, artificial
SAFYRYT

SEQ ID NO: 52 - protein, 9 aa, artificial
QQYYSIPWT

SEQ ID NO: 53 - protein, 5 aa, artificial
EYIMH

SEQ ID NO: 54 - protein, 17 aa, artificial
GINPNSGGTTYNEKFKG

SEQ ID NO: 55 - protein, 9 aa, artificial
RMPYWYFDV

SEQ ID NO: 56 - protein, 10 aa, artificial
SASSSVSYIH

SEQ ID NO: 57 - protein, 7 aa, artificial
DTSKLAS

SEQ ID NO: 58 - protein, 9 aa, artificial
QQWVSNPLT

SEQ ID NO: 59 - protein, 5 aa, artificial
EYIMH

SEQ ID NO: 60 - protein, 17 aa, artificial
GINPNTGGITYNQKFKD

SEQ ID NO: 61 - protein, 11 aa, artificial
AGGNFLWYFDV

SEQ ID NO: 62 - protein, 10 aa, artificial
SASSSVSYMH

SEQ ID NO: 63 - protein, 7 aa, artificial
DTSKLAS

SEQ ID NO: 64 - protein, 9 aa, artificial
QQWNSNPLT

SEQ ID NO: 65 - protein, 5 aa, artificial
SYDIN

SEQ ID NO: 66 - protein, 17 aa, artificial
WIDPGDGSTKYNEKFKG

SEQ ID NO: 67 - protein, 5 aa, artificial
RGFDY

SEQ ID NO: 68 - protein, 10 aa, artificial
RTSSSVSYLH

SEQ ID NO: 69 - protein, 7 aa, artificial
DTSNLAS

SEQ ID NO: 70 - protein, 9 aa, artificial
HQRSSYPWT

SEQ ID NO: 71 - protein, 5 aa, artificial
SYAVS

SEQ ID NO: 72 - protein, 17 aa, artificial
SISGGGIYIYYPDSVKG

SEQ ID NO: 73 - protein, 9 aa, artificial
HGGAGYFDY

SEQ ID NO: 74 - protein, 11 aa, artificial
RGSESVHSYLA

SEQ ID NO: 75 - protein, 7 aa, artificial
NAKTLQS

SEQ ID NO: 76 - protein, 10 aa, artificial
QQHYGSPPWT

SEQ ID NO: 77 - protein, 5 aa, artificial
DYAMH

SEQ ID NO: 78 - protein, 17 aa, artificial
VINSYYGNTHYNQKFKG

SEQ ID NO: 79 - protein, 17 aa, artificial
AGGYSYGSSYRPDRFAY

SEQ ID NO: 80 - protein, 11 aa, artificial
LASQTIGTWLA

SEQ ID NO: 81 - protein, 7 aa, artificial
AATNLAD

SEQ ID NO: 82 - protein, 9 aa, artificial
QQLYSTPYT

SEQ ID NO: 83 - protein, 5 aa, artificial
EYTMH

SEQ ID NO: 84 - protein, 17 aa, artificial
GINTDNGGTTYSQKFKD

SEQ ID NO: 85 - protein, 12 aa, artificial
SFNNYGPAWFAY

SEQ ID NO: 86 - protein, 11 aa, artificial
KASQDVRSAVA

SEQ ID NO: 87 - protein, 7 aa, artificial
WASTRHT

SEQ ID NO: 88 - protein, 8 aa, artificial
QQYSSYFT

SEQ ID NO: 89 - protein, 5 aa, artificial
ENTMH

SEQ ID NO: 90 - protein, 17 aa, artificial
GINPNNGGTTYNQKFKG

SEQ ID NO: 91 - protein, 12 aa, artificial
RGRWPPDWYFDV

SEQ ID NO: 92 - protein, 10 aa, artificial
SASSSLSYMH

SEQ ID NO: 93 - protein, 7 aa, artificial
DTSKLAS

SEQ ID NO: 94 - protein, 9 aa, artificial
QQWSSNPLT

SEQ ID NO: 95 - protein, 5 aa, artificial
SYYIY

SEQ ID NO: 96 - protein, 17 aa, artificial
GIKPSNGDTNFNAKFMN

SEQ ID NO: 97 - protein, 11 aa, artificial
FFYGSPYDFDV

SEQ ID NO: 98 - protein, 11 aa, artificial
KASENVDTHVS

SEQ ID NO: 99 - protein, 7 aa, artificial
GTSNRFT

SEQ ID NO: 100 - protein, 9 aa, artificial
GQSYRYPYT

SEQ ID NO: 101 - protein, 5 aa, artificial
EYVMH

SEQ ID NO: 102 - protein, 17 aa, artificial
GINPNTGGTTYNQKFEG

SEQ ID NO: 103 - protein, 11 aa, artificial
RMPFGISAMDY

SEQ ID NO: 104 - protein, 10 aa, artificial
SASSSVSYIH

SEQ ID NO: 105 - protein, 7 aa, artificial
ETSKLAS

SEQ ID NO: 106 - protein, 9 aa, artificial
HQWISYPPT

SEQ ID NO: 107 - protein, 5 aa, artificial
DHAIH

SEQ ID NO: 108 - protein, 17 aa, artificial
VINTYSGNTNFNQKLKG

SEQ ID NO: 109 - protein, 14 aa, artificial
GAHSSGYPYWYFDV

SEQ ID NO: 110 - protein, 10 aa, artificial
RASSSVSYMH

SEQ ID NO: 111 - protein, 7 aa, artificial
ATSNLAS

SEQ ID NO: 112 - protein, 9 aa, artificial
QQWSTNPFT

SEQ ID NO: 113 - protein, 118 aa, artificial
QVQLVQSGAEVKKPGASVKVSCKTSGYTFTEYIMHWVRQAPGQGLEWIGGINPNSGGTTYNEKFKGRATLTVDKSISTAYMELSRLRSDDTAVYYCARRMPYWYFDVWGQGTMVTVSS

SEQ ID NO: 114 - protein, 106 aa, artificial
EIVLTQSPATLSLSPGERATLSCSASSSVSYIHWYQQKPGQAPRRWVYDTSKLASGIPARFSGSGSGTDYTLTISSLEPEDFAVYYCQQWVSNPLTFGQGTKLEIK

SEQ ID NO: 115 - protein, 120 aa, artificial
QVQLVQSGAEVKKPGASVKVSCKTSGYTFTEYIMHWVRQAPGQGLEWIGGINPNTGGITYNQKFKDRATLTVDKSISTAYMELSRLRSDDTAVYYCARAGGNFLWYFDVWGQGTMVTVSS

SEQ ID NO: 116 - protein, 106 aa, artificial
EIVLTQSPATLSLSPGERATLSCSASSSVSYMHWYQQKPGQAPRRWLYDTSKLASGIPARFSGSGSGTDYTLTISSLEPEDFAVYYCQQWNSNPLTFGQGTKLEIK

SEQ ID NO: 117 - protein, 118 aa, artificial
QVQLVQSGAEVKKPGASVKVSCKASGYTFTEYTIHWVRQAPGQGLEWIGGINPNSGGTTYNLKFKGRATLTVDKSTSTVYMELSSLRSEDTAVYYCARKEGFFTTDYWGQGTLVTVSS

SEQ ID NO: 118 - protein, 106 aa, artificial
ETVLTQSPATLSLSPGERATLSCSASSSLSYIHWYQQKPGQAPRRWIYDTSNLATGIPARFSGSGSGTDYTLTISSLEPEDFAVYYCQQWHYNPPTFGGGTKVEIK

SEQ ID NO: 119 - protein, 114 aa, artificial
QVQLVQSGAEVKKPGASVKVSCKASGYTFTSYDINWVRQATGQGLEWIGWIDPGDGSTKYNEKFKGRATLTANKSISTAYMELSSLRSEDTAVYYCVRRGFDYWGQGTLVTVSS

SEQ ID NO: 120 - protein, 106 aa, artificial
EIVLTQSPATLSLSPGERATLSCRTSSSVSYLHWFQQKPGQAPRLWIHDTSNLASGFPARFSGSGSGTDYTLTISSLEPEDFAVYYCHQRSSYPWTFGGGTKVEIK

SEQ ID NO: 121 - protein, 121 aa, artificial
QVQLVQSGAEVKKPGSSVKVSCKASGYTFITYTIHWVRQAPGQGLEWIGYINPTSDYANFNQKFKDRATLTADKSTSTAYMELSSLRSEDTAVYYCARWGTTVFQFYFDYWGQGTLVTVSS

SEQ ID NO: 122 - protein, 106 aa, artificial
EIVLTQSPATLSLSPGERATLSCRASQSLSYINWYQQKPGKAPKPWIYATSSLQSGVPSRFSGSASGTDYTLTISSLQPEDFATYYCQHWSSDPPTIGGGTKVEIK

SEQ ID NO: 123 - protein, 118 aa, artificial
EVQLVESGGGLVKPGGSLRLSCAASGFTFSSYAVSWVRQAPGKGLEWVASISGGGIYIYYPDSVKGRFTISRDNAKNSLYLQMNSLRAEDTAVYYCARHGGAGYFDYWGQGTLVTVSS

SEQ ID NO: 124 - protein, 108 aa, artificial
DSQMTQSPSSLSASVGDRVTITCRGSESVHSYLAWYQQKPGKAPKLLVYNAKTLQSGVPSRFSGSGSGTDFTLTISSLQPEDFATYYCQQHYGSPPWTFGGGTKVEIK